European Patent Application EP 4 119 576 A1, published January 18, 2023. Title: A monoclonal antibody specifically binding to a sugar chain in which a terminal sialic acid residue is bound to galactose with an  ¿2,3 bond, and a method for measuring a sugar chain in which a terminal sialic acid residue is bound to galactose with an  ¿2,3 bond. Applicant: HIROSAKI UNIVERSITY SYSTEM INSTRUMENTS Co., Ltd. The sequence listing filed with the application follows.

SEQUENCE LISTING (16 sequences)

SEQ ID NO: 1 - protein, 9 aa, Oryctolagus cuniculus
GFDLSNNYV

SEQ ID NO: 2 - protein, 9 aa, Oryctolagus cuniculus
IYTGSSGSA

SEQ ID NO: 3 - protein, 19 aa, Oryctolagus cuniculus
ARGDVFTRGGVEYAGVMTL

SEQ ID NO: 4 - protein, 6 aa, Oryctolagus cuniculus
QSISTA

SEQ ID NO: 5 - protein, 3 aa, Oryctolagus cuniculus
SAS

SEQ ID NO: 6 - protein, 13 aa, Oryctolagus cuniculus
QGYDYIHSRADNA

SEQ ID NO: 7 - protein, 9 aa, Oryctolagus cuniculus
GFSFSGSDW

SEQ ID NO: 8 - protein, 9 aa, Oryctolagus cuniculus
IYAGSSGRT

SEQ ID NO: 9 - protein, 6 aa, Oryctolagus cuniculus
EREVDL

SEQ ID NO: 10 - protein, 7 aa, Oryctolagus cuniculus
QSVYSNY

SEQ ID NO: 11 - protein, 3 aa, Oryctolagus cuniculus
QAS

SEQ ID NO: 12 - protein, 11 aa, Oryctolagus cuniculus
QGAYSSGDGRA

SEQ ID NO: 13 - protein, 125 aa, Oryctolagus cuniculus
QEQLEESGGDLVKPEGSLTLTCTASGFDLSNNYVMCWVRQAPGKGLEWIACIYTGSSGSAYYASWPKGRFTISKTSSTTVTLQMTSLTAADTATYFCARGDVFTRGGVEYAGVMTLWGPGTLVTV

SEQ ID NO: 14 - protein, 114 aa, Oryctolagus cuniculus
ARCALVMTQTASPVEAAVGGTVTIKCQASQSISTALAWYQQKPGQPPKLLIYSASKLASGVPSRFSGSGSGTEFTLTISGVQCDDAATYYCQGYDYIHSRADNAFGGGTEVVVK

SEQ ID NO: 15 - protein, 113 aa, Oryctolagus cuniculus
RSLEESGGDLVKPGASLTLTCTASGFSFSGSDWISWVRQAPGKGLEWIAYIYAGSSGRTRYASWAKGRFTISKTSSTTVTLQMTSLTAADTATYFCEREVDLWGPGTLVTVSS

SEQ ID NO: 16 - protein, 113 aa, Oryctolagus cuniculus
ATFAQVVTQTPSPVSATLGGTVTINCQSSQSVYSNYLSWFQQQPGQPPKLLMYQASNLASGVPSRFKGSGSGTQFTLTISSVQCDDAATYYCQGAYSSGDGRAFGGGTEVVVK